European Patent Application EP 4 141 020 A1, published March 1, 2023. Title: Novel cell penetrating peptides and use thereof. Applicant: Imnewrun Biosciences, Inc. The sequence listing filed with the application follows.

SEQUENCE LISTING (12 sequences)

SEQ ID NO: 1 - protein, 16 aa, Artificial Sequence
  transpep-1
GHHERLKSDEWSVTSG

SEQ ID NO: 2 - protein, 16 aa, Artificial Sequence
  transpep-2
GHHERLKSAEWSVTSG

SEQ ID NO: 3 - protein, 16 aa, Artificial Sequence
  transpep-3
GHHERLKSDAWSVTSG

SEQ ID NO: 4 - protein, 16 aa, Artificial Sequence
  transpep-4
GHHERLKSDEWAVTSG

SEQ ID NO: 5 - protein, 16 aa, Artificial Sequence
  transpep-5
GHHERLKSAAWSVTSG

SEQ ID NO: 6 - protein, 16 aa, Artificial Sequence
  transpep-6
GHHERLKSAEWAVTSG

SEQ ID NO: 7 - protein, 16 aa, Artificial Sequence
  transpep-7
GHHERLKSDAWAVTSG

SEQ ID NO: 8 - protein, 16 aa, Artificial Sequence
  transpep-8
GHHERLKSEEWSVTSG

SEQ ID NO: 9 - protein, 16 aa, Artificial Sequence
  transpep-9
GHHERLKSYEWSVTSG

SEQ ID NO: 10 - protein, 16 aa, Artificial Sequence
  transpep-10
GHHERLKSDDWSVTSG

SEQ ID NO: 11 - protein, 16 aa, Artificial Sequence
  transpep-11
GHHERLKSDYWSVTSG

SEQ ID NO: 12 - protein, 16 aa, Artificial Sequence
  transpep-12
GHHERLKSDEWNVTSG